European Patent Application EP 4 585 619 A1, published July 16, 2025. Title: anti-VISTA monoclonal antibody and uses thereof. Applicant: 주식회사 시클리드. Application KR. The sequence listing filed with the application follows.

SEQUENCE LISTING (72 sequences)

SEQ ID NO: 1 - protein, 5 aa, synthetic construct
SYWIA

SEQ ID NO: 2 - protein, 17 aa, synthetic construct
TISGSGGYTYYAESVKG

SEQ ID NO: 3 - protein, 9 aa, synthetic construct
RDSSGWLNY

SEQ ID NO: 4 - protein, 11 aa, synthetic construct
RASQSITSHLA

SEQ ID NO: 5 - protein, 7 aa, synthetic construct
DASNRAT

SEQ ID NO: 6 - protein, 10 aa, synthetic construct
QQYNNWPPIT

SEQ ID NO: 7 - protein, 447 aa, synthetic construct
EVQLLESGGGLVQPGGSLRLSCAASGFTFSSYWIAWVRQAPGKGLEWVSTISGSGGYTYYAESVKGRFTISRDNSKNTLYLQMNSLRAEDTAVYYCARDSSGWLNYWGQGTLVTVSSASTKGPSVFPLAPSSKSTSGGTAALGCLVKDYFPEPVTVSWNSGALTSGVHTFPAVLQSSGLYSLSSVVTVPSSSLGTQTYICNVNHKPSNTKVDKKVEPKSCDKTHTCPPCPAPELLGGPSVFLFPPKPKDTLMISRTPEVTCVVVDVSHEDPEVKFNWYVDGVEVHNAKTKPREEQYNSTYRVVSVLTVLHQDWLNGKEYKCKVSNKALPAPIEKTISKAKGQPREPQVYTLPPSRDELTKNQVSLTCLVKGFYPSDIAVEWESNGQPENNYKTTPPVLDSDGSFFLYSKLTVDKSRWQQGNVFSCSVMHEALHNHYTQKSLSLSPGK

SEQ ID NO: 8 - protein, 215 aa, synthetic construct
EIVLTQSPGTLSLSPGERATLSCRASQSITSHLAWYQQKPGQAPRLLIYDASNRATGIPDRFSGSGSGTDFTLTISRLEPEDFAVYYCQQYNNWPPITFGQGTKVEIKRTVAAPSVFIFPPSDEQLKSGTASVVCLLNNFYPREAKVQWKVDNALQSGNSQESVTEQDSKDSTYSLSSTLTLSKADYEKHKVYACEVTHQGLSSPVTKSFNRGEC

SEQ ID NO: 9 - protein, 5 aa, synthetic construct
DYYMH

SEQ ID NO: 10 - protein, 17 aa, synthetic construct
EIIPIFDTANYAQKFQD

SEQ ID NO: 11 - protein, 9 aa, synthetic construct
RSTGDYFDY

SEQ ID NO: 12 - protein, 11 aa, synthetic construct
SGDKLGNKYTS

SEQ ID NO: 13 - protein, 7 aa, synthetic construct
DNNKRPS

SEQ ID NO: 14 - protein, 11 aa, synthetic construct
GTWDSSLSAYV

SEQ ID NO: 15 - protein, 447 aa, synthetic construct
EVQLLESGGGLVQPGGSLRLSCAASGFTFSDYYMHWVRQAPGKGLEWVSEIIPIFDTANYAQKFQDRFTISRDNSKNTLYLQMNSLRAEDTAVYYCARSTGDYFDYWGQGTLVTVSSASTKGPSVFPLAPSSKSTSGGTAALGCLVKDYFPEPVTVSWNSGALTSGVHTFPAVLQSSGLYSLSSVVTVPSSSLGTQTYICNVNHKPSNTKVDKKVEPKSCDKTHTCPPCPAPELLGGPSVFLFPPKPKDTLMISRTPEVTCVVVDVSHEDPEVKFNWYVDGVEVHNAKTKPREEQYNSTYRVVSVLTVLHQDWLNGKEYKCKVSNKALPAPIEKTISKAKGQPREPQVYTLPPSRDELTKNQVSLTCLVKGFYPSDIAVEWESNGQPENNYKTTPPVLDSDGSFFLYSKLTVDKSRWQQGNVFSCSVMHEALHNHYTQKSLSLSPGK

SEQ ID NO: 16 - protein, 215 aa, synthetic construct
QSVLTQPPSASGTPGQRVTISCSGDKLGNKYTSWYQQLPGTAPKLLIYDNNKRPSGVPDRFSGSKSGTSASLAISGLRSEDEADYYCGTWDSSLSAYVFGGGTKLTVLRTVAAPSVFIFPPSDEQLKSGTASVVCLLNNFYPREAKVQWKVDNALQSGNSQESVTEQDSKDSTYSLSSTLTLSKADYEKHKVYACEVTHQGLSSPVTKSFNRGEC

SEQ ID NO: 17 - protein, 5 aa, synthetic construct
EKSIH

SEQ ID NO: 18 - protein, 17 aa, synthetic construct
GTSANTGNTYYADSVKG

SEQ ID NO: 19 - protein, 10 aa, synthetic construct
HHNWAGYFDY

SEQ ID NO: 20 - protein, 11 aa, synthetic construct
QASHAISNYIN

SEQ ID NO: 21 - protein, 7 aa, synthetic construct
DASNRAT

SEQ ID NO: 22 - protein, 9 aa, synthetic construct
QQSNSFPYT

SEQ ID NO: 23 - protein, 448 aa, synthetic construct
EVQLLESGGGLVQPGGSLRLSCVASGFTFSEKSIHWVRQAPGKGLEWVSGTSANTGNTYYADSVKGRFTISRDNSKNTLYLQMNSLRAEDTAVYYCAHHNWAGYFDYWGQGTLVTVSSASTKGPSVFPLAPSSKSTSGGTAALGCLVKDYFPEPVTVSWNSGALTSGVHTFPAVLQSSGLYSLSSVVTVPSSSLGTQTYICNVNHKPSNTKVDKKVEPKSCDKTHTCPPCPAPELLGGPSVFLFPPKPKDTLMISRTPEVTCVVVDVSHEDPEVKFNWYVDGVEVHNAKTKPREEQYNSTYRVVSVLTVLHQDWLNGKEYKCKVSNKALPAPIEKTISKAKGQPREPQVYTLPPSRDELTKNQVSLTCLVKGFYPSDIAVEWESNGQPENNYKTTPPVLDSDGSFFLYSKLTVDKSRWQQGNVFSCSVMHEALHNHYTQKSLSLSPGK

SEQ ID NO: 24 - protein, 214 aa, synthetic construct
EIVLTQSPGILSLSPGERATLSCQASHAISNYINWYQQKPGQAPRLLIYDASNRATGIPDRFSGSGSGTDFTLTISRLEPEDFAVYYCQQSNSFPYTFGQGTKVEIKRTVAAPSVFIFPPSDEQLKSGTASVVCLLNNFYPREAKVQWKVDNALQSGNSQESVTEQDSKDSTYSLSSTLTLSKADYEKHKVYACEVTHQGLSSPVTKSFNRGEC

SEQ ID NO: 25 - protein, 5 aa, synthetic construct
TAWMS

SEQ ID NO: 26 - protein, 17 aa, synthetic construct
RVNPSDSHTDYSPSFQD

SEQ ID NO: 27 - protein, 10 aa, synthetic construct
RVPPGYGFDI

SEQ ID NO: 28 - protein, 11 aa, synthetic construct
QASQDITNYLN

SEQ ID NO: 29 - protein, 7 aa, synthetic construct
DASNRAT

SEQ ID NO: 30 - protein, 9 aa, synthetic construct
QQSYSTPFT

SEQ ID NO: 31 - protein, 448 aa, synthetic construct
EVQLLESGGGLVQPGGSLRLSCAASGFTFSTAWMSWVRQAPGKGLEWVSRVNPSDSHTDYSPSFQDRFTISRDNSKNTLYLQMNSLRAEDTAVYYCARVPPGYGFDIWGQGTLVTVSSASTKGPSVFPLAPSSKSTSGGTAALGCLVKDYFPEPVTVSWNSGALTSGVHTFPAVLQSSGLYSLSSVVTVPSSSLGTQTYICNVNHKPSNTKVDKKVEPKSCDKTHTCPPCPAPELLGGPSVFLFPPKPKDTLMISRTPEVTCVVVDVSHEDPEVKFNWYVDGVEVHNAKTKPREEQYNSTYRVVSVLTVLHQDWLNGKEYKCKVSNKALPAPIEKTISKAKGQPREPQVYTLPPSRDELTKNQVSLTCLVKGFYPSDIAVEWESNGQPENNYKTTPPVLDSDGSFFLYSKLTVDKSRWQQGNVFSCSVMHEALHNHYTQKSLSLSPGK

SEQ ID NO: 32 - protein, 214 aa, synthetic construct
EIVLTQSPGTLSLSPGERATLSCQASQDITNYLNWYQQKPGQAPRLLIYDASNRATGIPDRFSGSGSGTDFTLTISRLEPEDFAVYYCQQSYSTPFTFGQGTKVEIKRTVAAPSVFIFPPSDEQLKSGTASVVCLLNNFYPREAKVQWKVDNALQSGNSQESVTEQDSKDSTYSLSSTLTLSKADYEKHKVYACEVTHQGLSSPVTKSFNRGEC

SEQ ID NO: 33 - protein, 5 aa, synthetic construct
NYAMS

SEQ ID NO: 34 - protein, 16 aa, synthetic construct
EISHSGTTNYNPSLKS

SEQ ID NO: 35 - protein, 9 aa, synthetic construct
TRAIWGFDY

SEQ ID NO: 36 - protein, 11 aa, synthetic construct
SRENIGSRSVH

SEQ ID NO: 37 - protein, 7 aa, synthetic construct
DNNERAS

SEQ ID NO: 38 - protein, 9 aa, synthetic construct
QAWDSSTAV

SEQ ID NO: 39 - protein, 445 aa, synthetic construct
EVQLLESGGGLVQPGGSLRLSCAASGFTFSNYAMSWVRQAPGKGLEWVSEISHSGTTNYNPSLKSRFTISRDNSKNTLYLQMNSLRAEDTAVYYCTRAIWGFDYWGQGTLVTVSSASTKGPSVFPLAPSSKSTSGGTAALGCLVKDYFPEPVTVSWNSGALTSGVHTFPAVLQSSGLYSLSSVVTVPSSSLGTQTYICNVNHKPSNTKVDKKVEPKSCDKTHTCPPCPAPELLGGPSVFLFPPKPKDTLMISRTPEVTCVVVDVSHEDPEVKFNWYVDGVEVHNAKTKPREEQYNSTYRVVSVLTVLHQDWLNGKEYKCKVSNKALPAPIEKTISKAKGQPREPQVYTLPPSRDELTKNQVSLTCLVKGFYPSDIAVEWESNGQPENNYKTTPPVLDSDGSFFLYSKLTVDKSRWQQGNVFSCSVMHEALHNHYTQKSLSLSPGK

SEQ ID NO: 40 - protein, 213 aa, synthetic construct
QSVLTQPPSASGTPGQRVTISCSRENIGSRSVHWYQQLPGTAPKLLIYDNNERASGVPNRFSGSKSGTSASLAISGLRSEDEADYYCQAWDSSTAVFGGGTKLTVLRTVAAPSVFIFPPSDEQLKSGTASVVCLLNNFYPREAKVQWKVDNALQSGNSQESVTEQDSKDSTYSLSSTLTLSKADYEKHKVYACEVTHQGLSSPVTKSFNRGEC

SEQ ID NO: 41 - protein, 5 aa, synthetic construct
NYYMH

SEQ ID NO: 42 - protein, 16 aa, synthetic construct
SISFTGSTSYNPSLKS

SEQ ID NO: 43 - protein, 12 aa, synthetic construct
RLGIPFFTYLDY

SEQ ID NO: 44 - protein, 11 aa, synthetic construct
GGNNIGSKSVH

SEQ ID NO: 45 - protein, 7 aa, synthetic construct
EDTERPS

SEQ ID NO: 46 - protein, 9 aa, synthetic construct
QAWDSSTVV

SEQ ID NO: 47 - protein, 449 aa, synthetic construct
EVQLLESGGGLVQPGGSLRLSCAASGFTFSNYYMHWVRQAPGKGLEWVSSISFTGSTSYNPSLKSRFTISRDNSKNTLYLQMNSLRAEDTAVYYCARLGIPFFTYLDYWGQGTLVTVSSASTKGPSVFPLAPSSKSTSGGTAALGCLVKDYFPEPVTVSWNSGALTSGVHTFPAVLQSSGLYSLSSVVTVPSSSLGTQTYICNVNHKPSNTKVDKKVEPKSCDKTHTCPPCPAPELLGGPSVFLFPPKPKDTLMISRTPEVTCVVVDVSHEDPEVKFNWYVDGVEVHNAKTKPREEQYNSTYRVVSVLTVLHQDWLNGKEYKCKVSNKALPAPIEKTISKAKGQPREPQVYTLPPSRDELTKNQVSLTCLVKGFYPSDIAVEWESNGQPENNYKTTPPVLDSDGSFFLYSKLTVDKSRWQQGNVFSCSVMHEALHNHYTQKSLSLSPGK

SEQ ID NO: 48 - protein, 213 aa, synthetic construct
QSVLTQPPSASGTPGQRVTISCGGNNIGSKSVHWYQQLPGTAPKLLIYEDTERPSGVSDRFSGSKSGTSASLAISGLRSEDEADYYCQAWDSSTVVFGGGTKLTVLRTVAAPSVFIFPPSDEQLKSGTASVVCLLNNFYPREAKVQWKVDNALQSGNSQESVTEQDSKDSTYSLSSTLTLSKADYEKHKVYACEVTHQGLSSPVTKSFNRGEC

SEQ ID NO: 49 - DNA, 92 bp, synthetic construct
  source 1..92: mol_type = other DNA
attcgatcgatatggagacagacacactcctgctatgggtactgctgctctgggttccaggttccacgtgggaaatcgtgctgacccagagc

SEQ ID NO: 50 - DNA, 33 bp, synthetic construct
  source 1..33: mol_type = other DNA
agccaccgtacgtttgatttccactttagtgcc

SEQ ID NO: 51 - DNA, 92 bp, synthetic construct
  source 1..92: mol_type = other DNA
attcgatcgatatggagacagacacactcctgctatgggtactgctgctctgggttccaggttccacgtgggaagtgcagctgctggaaagt

SEQ ID NO: 52 - DNA, 33 bp, synthetic construct
  source 1..33: mol_type = other DNA
cttggtgctagcgctgctcacggtcaccagagt

SEQ ID NO: 53 - DNA, 92 bp, synthetic construct; identical to SEQ ID NO: 49
  source 1..92: mol_type = other DNA

SEQ ID NO: 54 - DNA, 33 bp, synthetic construct; identical to SEQ ID NO: 50
  source 1..33: mol_type = other DNA

SEQ ID NO: 55 - DNA, 92 bp, synthetic construct; identical to SEQ ID NO: 51
  source 1..92: mol_type = other DNA

SEQ ID NO: 56 - DNA, 33 bp, synthetic construct; identical to SEQ ID NO: 52
  source 1..33: mol_type = other DNA

SEQ ID NO: 57 - DNA, 92 bp, synthetic construct; identical to SEQ ID NO: 49
  source 1..92: mol_type = other DNA

SEQ ID NO: 58 - DNA, 33 bp, synthetic construct; identical to SEQ ID NO: 50
  source 1..33: mol_type = other DNA

SEQ ID NO: 59 - DNA, 92 bp, synthetic construct; identical to SEQ ID NO: 51
  source 1..92: mol_type = other DNA

SEQ ID NO: 60 - DNA, 33 bp, synthetic construct; identical to SEQ ID NO: 52
  source 1..33: mol_type = other DNA

SEQ ID NO: 61 - DNA, 92 bp, synthetic construct; identical to SEQ ID NO: 49
  source 1..92: mol_type = other DNA

SEQ ID NO: 62 - DNA, 33 bp, synthetic construct; identical to SEQ ID NO: 50
  source 1..33: mol_type = other DNA

SEQ ID NO: 63 - DNA, 92 bp, synthetic construct; identical to SEQ ID NO: 51
  source 1..92: mol_type = other DNA

SEQ ID NO: 64 - DNA, 33 bp, synthetic construct; identical to SEQ ID NO: 52
  source 1..33: mol_type = other DNA

SEQ ID NO: 65 - DNA, 92 bp, synthetic construct; identical to SEQ ID NO: 49
  source 1..92: mol_type = other DNA

SEQ ID NO: 66 - DNA, 33 bp, synthetic construct; identical to SEQ ID NO: 50
  source 1..33: mol_type = other DNA

SEQ ID NO: 67 - DNA, 92 bp, synthetic construct; identical to SEQ ID NO: 51
  source 1..92: mol_type = other DNA

SEQ ID NO: 68 - DNA, 33 bp, synthetic construct; identical to SEQ ID NO: 52
  source 1..33: mol_type = other DNA

SEQ ID NO: 69 - DNA, 92 bp, synthetic construct; identical to SEQ ID NO: 49
  source 1..92: mol_type = other DNA

SEQ ID NO: 70 - DNA, 33 bp, synthetic construct; identical to SEQ ID NO: 50
  source 1..33: mol_type = other DNA

SEQ ID NO: 71 - DNA, 92 bp, synthetic construct; identical to SEQ ID NO: 51
  source 1..92: mol_type = other DNA

SEQ ID NO: 72 - DNA, 33 bp, synthetic construct; identical to SEQ ID NO: 52
  source 1..33: mol_type = other DNA